European Patent Application EP 4 591 884 A1, published July 30, 2025. Title: 用于核酸递送的脂质化合物以及包含所述脂质化合物的相关应用及药物. Applicant: 中国医学科学院基础医学研究所. Application CN. The sequence listing filed with the application follows.

SEQUENCE LISTING (1 sequence)

SEQ ID NO: 1 - RNA, 25 nt, synthetic construct
  source 1..25: mol_type = other RNA
tccggaatgattgggcgtaaagcgt